European Patent Application EP 4 674 871 A1, published January 7, 2026. Title: 接着性及び機能性を有する組換えタンパク質及びそれを含む組成物. Applicant: 株式会社ノベルジェン. The sequence listing filed with the application follows.

SEQUENCE LISTING (80 sequences)

SEQ ID NO: 1 - protein, 37 aa, Mytilus galloprovincialis derived FP2-motif (variant 1)
PVNPCLKKPCKYNGVCKPRGGSYKCFCKGGYYGYNCN

SEQ ID NO: 2 - protein, 36 aa, Mytilus galloprovincialis derived FP2-motif (variant 2)
LKNACKPNQCKNKSRCVPVGKTFKCVCRNGNFGRLC

SEQ ID NO: 3 - protein, 37 aa, Mytilus galloprovincialis derived FP2-motif (variant 3)
EKNVCSPNPCKNNGKCSPLGKTGYKCTCSGGYTGPRC

SEQ ID NO: 4 - protein, 37 aa, Mytilus galloprovincialis derived FP2-motif (variant 4)
EVHACKPNPCKNKGRCFPDGKTGYKCRCVDGYSGPTC

SEQ ID NO: 5 - protein, 37 aa, Mytilus galloprovincialis derived FP2-motif (variant 5)
QENACKPNPCSNGGTCSADKFGDYSCECRPGYFGPEC

SEQ ID NO: 6 - protein, 37 aa, Mytilus galloprovincialis derived FP2-motif (variant 6)
ERYVCAPNPCKNGGICSSDGSGGYRCRCKGGYSGPTC

SEQ ID NO: 7 - protein, 36 aa, Mytilus galloprovincialis derived FP2-motif (variant 7)
KVNVCKPTPCKNSGRCVNKGSSYNCICKGGYSGPTC

SEQ ID NO: 8 - protein, 39 aa, Mytilus galloprovincialis derived FP2-motif (variant 8)
GENVCKPNPCQNRGRCYPDNSDDGFKCRCVGGYKGPTCE

SEQ ID NO: 9 - protein, 38 aa, Mytilus galloprovincialis derived FP2-motif (variant 9)
DKPNPCNTKPCKNGGKCNYNGKIYTCKCAYGWRGRHCT

SEQ ID NO: 10 - protein, 42 aa, Mytilus galloprovincialis derived FP2-motif (variant 10)
DKAYKPNPCVVSKPCKNRGKCIWNGKAYRCKCAYGYGGRHCT

SEQ ID NO: 11 - protein, 41 aa, Mytilus galloprovincialis derived FP2-motif (variant 11)
KKSYKKNPCASRPCKNRGKCTDKGNGYVCKCARGYSGRYCS

SEQ ID NO: 12 - protein, 53 aa, human derived EGF
NSDSECPLSHDGYCLHDGVCMYIEALDKYACNCVVGYIGERCQYRDLKWWELR

SEQ ID NO: 13 - protein, 10 aa, Mytilus galloprovincialis derived FP1-motif (variant 1)
AKPTYPSTYK

SEQ ID NO: 14 - protein, 10 aa, Mytilus galloprovincialis derived FP1-motif (variant 2)
AKPSYPPTYK

SEQ ID NO: 15 - protein, 9 aa, Mytilus galloprovincialis derived FP1-motif (variant 2-1)
AKPSYPPTY

SEQ ID NO: 16 - protein, 10 aa, Mytilus galloprovincialis derived FP1-motif (variant 3)
AKPSYPSTYK

SEQ ID NO: 17 - protein, 10 aa, Mytilus galloprovincialis derived FP1-motif (variant 4)
AKSSYPPTYK

SEQ ID NO: 18 - protein, 60 aa, 6 repeated FP1-motif(variant 1)
AKPTYPSTYKAKPSYPPTYKAKPSYPSTYKAKSSYPPTYKAKPSYPPTYKAKPSYPPTYK

SEQ ID NO: 19 - protein, 59 aa, 6 repeated FP1-motif(variant 1-1)
AKPTYPSTYKAKPSYPPTYKAKPSYPSTYKAKSSYPPTYKAKPSYPPTYKAKPSYPPTY

SEQ ID NO: 20 - protein, 30 aa, 3 repeated FP1-motif(variant 1)
AKSSYPPTYKAKPSYPPTYKAKPSYPPTYK

SEQ ID NO: 21 - protein, 30 aa, 3 repeated FP1-motif(variant 2)
AKPTYPSTYKAKPSYPPTYKAKPSYPSTYK

SEQ ID NO: 22 - protein, 90 aa, 9 repeated FP1-motif(variant 1)
AKPTYPSTYKAKPSYPPTYKAKPSYPSTYKAKPTYPSTYKAKPSYPPTYKAKPSYPSTYKAKSSYPPTYKAKPSYPPTYKAKPSYPPTYK

SEQ ID NO: 23 - protein, 90 aa, 9 repeated FP1-motif(variant 2)
AKPTYPSTYKAKPSYPPTYKAKPSYPSTYKAKSSYPPTYKAKPSYPPTYKAKPSYPPTYKAKSSYPPTYKAKPSYPPTYKAKPSYPPTYK

SEQ ID NO: 24 - protein, 10 aa, Ca combined domain
CVNKGSSYNC

SEQ ID NO: 25 - DNA, 480 bp, synthetic construct(FP121-6 (prototype) gene (gene fragment after synthesis))
  source 1..480: mol_type = other DNA
catatggctaaaccaacatatccctcaacttacaaggcgaagccgtcctacccgcctacttacaaggctaagccgtcttacccgtccacctacaaagctaagagcagctacccgccaacgtacaaagcgaaaccgagctatccgccgacgtacaaggccaagccgtcctacccgcctacctataaacccgtgaacccgtgtctgaaaaaaccgtgcaaatataacggcgtttgtaaaccgcgtggtggcagctacaagtgcttctgcaaaggtggttattacggctataactgcaatgcaaagccgacctacccgtcaacctataaggccaagccgagttatccaccgacctataaggcgaagccgagctatccgtcgacctacaaggcgaaaagcagctacccaccgacctataaagcgaaaccgagctatccgccgacctataaggcaaaaccgtcttacccgccgacgtacctcgag

SEQ ID NO: 26 - DNA, 473 bp, FP121-6 (prototype) gene (gene fragment after vector insertion)
  source 1..473: mol_type = genomic DNA
tatggctaaaccaacatatccctcaacttacaaggcgaagccgtcctacccgcctacttacaaggctaagccgtcttacccgtccacctacaaagctaagagcagctacccgccaacgtacaaagcgaaaccgagctatccgccgacgtacaaggccaagccgtcctacccgcctacctataaacccgtgaacccgtgtctgaaaaaaccgtgcaaatataacggcgtttgtaaaccgcgtggtggcagctacaagtgcttctgcaaaggtggttattacggctataactgcaatgcaaagccgacctacccgtcaacctataaggccaagccgagttatccaccgacctataaggcgaagccgagctatccgtcgacctacaaggcgaaaagcagctacccaccgacctataaagcgaaaccgagctatccgccgacctataaggcaaaaccgtcttacccgccgacgtacc

SEQ ID NO: 27 - DNA, 20 bp, synthetic construct(T7promoter-1 Forward primer)
  source 1..20: mol_type = other DNA
taatacgactcactataggg

SEQ ID NO: 28 - DNA, 41 bp, synthetic construct(FP121-6 gene reverse primer)
  source 1..41: mol_type = other DNA
tttctcgagttacttgtacgtcggcgggtaagacggttttg

SEQ ID NO: 29 - DNA, 574 bp, synthetic construct(FP121-6 gene (gene fragment after synthesis))
  source 1..574: mol_type = other DNA
taatacgactcactataggggaattgtgagcggataacaattcccctctagaaataattttgtttaactttaagaaggagatatacatatggctaaaccaacatatccctcaacttacaaggcgaagccgtcctacccgcctacttacaaggctaagccgtcttacccgtccacctacaaagctaagagcagctacccgccaacgtacaaagcgaaaccgagctatccgccgacgtacaaggccaagccgtcctacccgcctacctataaacccgtgaacccgtgtctgaaaaaaccgtgcaaatataacggcgtttgtaaaccgcgtggtggcagctacaagtgcttctgcaaaggtggttattacggctataactgcaatgcaaagccgacctacccgtcaacctataaggccaagccgagttatccaccgacctataaggcgaagccgagctatccgtcgacctacaaggcgaaaagcagctacccaccgacctataaagcgaaaccgagctatccgccgacctataaggcaaaaccgtcttacccgccgacgtacaagtaactcgagaaa

SEQ ID NO: 30 - DNA, 479 bp, synthetic construct(FP121-6 gene (gene fragment after vector insertion))
  source 1..479: mol_type = other DNA
tatggctaaaccaacatatccctcaacttacaaggcgaagccgtcctacccgcctacttacaaggctaagccgtcttacccgtccacctacaaagctaagagcagctacccgccaacgtacaaagcgaaaccgagctatccgccgacgtacaaggccaagccgtcctacccgcctacctataaacccgtgaacccgtgtctgaaaaaaccgtgcaaatataacggcgtttgtaaaccgcgtggtggcagctacaagtgcttctgcaaaggtggttattacggctataactgcaatgcaaagccgacctacccgtcaacctataaggccaagccgagttatccaccgacctataaggcgaagccgagctatccgtcgacctacaaggcgaaaagcagctacccaccgacctataaagcgaaaccgagctatccgccgacctataaggcaaaaccgtcttacccgccgacgtacaagtaac

SEQ ID NO: 31 - DNA, 483 bp, synthetic construct(cbFP121-6 gene (gene fragment after synthesis))
  source 1..483: mol_type = other DNA
catatggctaaaccaacttacccctcaacatataaggcgaaaccgtcctacccgccgacatacaaagcaaagccgtcttacccgtcgacctacaaagcgaaatccagctatccgcctacctacaaggcgaaaccgagctatccaccgacctataaagccaagccatcttacccgccgacctataagaaagtcaacgtgtgcaaaccgactccgtgtaaaaacagcggtcgttgtgttaataaaggtagcagctataactgcatctgcaaaggcggttatagcggccctacgtgcgcaaaaccgacctatccgtcgacctacaaggctaagccgtcctatccgccgacctacaaggctaaaccgtcttacccgtccacctataaggcgaagagcagctacccgccaacgtacaaagcgaagccgtcatacccgccaacgtacaaggccaagccgagctatccgccgacctacaagtaactcgag

SEQ ID NO: 32 - DNA, 476 bp, synthetic construct(cbFP121-6 gene (gene fragment after vector insertion))
  source 1..476: mol_type = other DNA
tatggctaaaccaacttacccctcaacatataaggcgaaaccgtcctacccgccgacatacaaagcaaagccgtcttacccgtcgacctacaaagcgaaatccagctatccgcctacctacaaggcgaaaccgagctatccaccgacctataaagccaagccatcttacccgccgacctataagaaagtcaacgtgtgcaaaccgactccgtgtaaaaacagcggtcgttgtgttaataaaggtagcagctataactgcatctgcaaaggcggttatagcggccctacgtgcgcaaaaccgacctatccgtcgacctacaaggctaagccgtcctatccgccgacctacaaggctaaaccgtcttacccgtccacctataaggcgaagagcagctacccgccaacgtacaaagcgaagccgtcatacccgccaacgtacaaggccaagccgagctatccgccgacctacaagtaac

SEQ ID NO: 33 - DNA, 534 bp, synthetic construct(hEGF-FP1-6 gene (gene fragment after synthesis))
  source 1..534: mol_type = other DNA
catatggctaaaccaacatatccctcaacttacaaggctaaaccgtcttacccgccgacgtacaaggccaaaccgagttatccgtcgacctataaggcgaagagcagctacccgccaacgtacaaggcgaaaccgtcctacccgccaacctacaaagccaagccgtcctacccgccaacctataagaacagcgacagcgagtgcccgctcagccacgacggctactgcctgcatgacggcgtttgtatgtatatcgaggcactggataaatatgcatgtaattgcgtcgtgggttatattggtgaacgttgccagtatcgtgatctgaaatggtgggaattgcgcgcaaagccgacttacccgagcacctacaaagcgaaaccgagctatccgccaacctacaaggctaaaccgagctatccgtcgacctataaagcgaaatccagctatccgccgacctacaaggcgaagccgtcatacccgcctacgtacaaagcgaagccgtcttatccgccgacctacaagtaactcgag

SEQ ID NO: 34 - DNA, 527 bp, synthetic construct(hEGF-FP1-6 gene (gene fragment after vector insertion))
  source 1..527: mol_type = other DNA
tatggctaaaccaacatatccctcaacttacaaggctaaaccgtcttacccgccgacgtacaaggccaaaccgagttatccgtcgacctataaggcgaagagcagctacccgccaacgtacaaggcgaaaccgtcctacccgccaacctacaaagccaagccgtcctacccgccaacctataagaacagcgacagcgagtgcccgctcagccacgacggctactgcctgcatgacggcgtttgtatgtatatcgaggcactggataaatatgcatgtaattgcgtcgtgggttatattggtgaacgttgccagtatcgtgatctgaaatggtgggaattgcgcgcaaagccgacttacccgagcacctacaaagcgaaaccgagctatccgccaacctacaaggctaaaccgagctatccgtcgacctataaagcgaaatccagctatccgccgacctacaaggcgaagccgtcatacccgcctacgtacaaagcgaagccgtcttatccgccgacctacaagtaac

SEQ ID NO: 35 - DNA, 192 bp, synthetic construct(FP121-1 gene (gene fragment after synthesis))
  source 1..192: mol_type = other DNA
aaacatatggccaagccgtcctacccgcctacctataaacccgtgaacccgtgtctgaaaaaaccgtgcaaatataacggcgtttgtaaaccgcgtggtggcagctacaagtgcttctgcaaaggtggttattacggctataactgcaatgcaaagccgacctacccgtcaacctataagtaactcgagaaa

SEQ ID NO: 36 - DNA, 179 bp, synthetic constructFP121-1 gene (gene fragment after vector insertion)
  source 1..179: mol_type = other DNA
tatggccaagccgtcctacccgcctacctataaacccgtgaacccgtgtctgaaaaaaccgtgcaaatataacggcgtttgtaaaccgcgtggtggcagctacaagtgcttctgcaaaggtggttattacggctataactgcaatgcaaagccgacctacccgtcaacctataagtaac

SEQ ID NO: 37 - DNA, 48 bp, synthetic construct(FP121-1 gene Forward primer)
  source 1..48: mol_type = other DNA
aaacatatggccaagccgtcctacccgcctacctataaacccgtgaac

SEQ ID NO: 38 - DNA, 47 bp, synthetic construct(FP121-1 gene reverse primer)
  source 1..47: mol_type = other DNA
tttctcgagttacttataggttgacgggtaggtcggctttgcattgc

SEQ ID NO: 39 - DNA, 312 bp, synthetic construct(FP121-3 gene (gene fragment after synthesis))
  source 1..312: mol_type = other DNA
aaacatatggctaagagcagctacccgccaacgtacaaagcgaaaccgagctatccgccgacgtacaaggccaagccgtcctacccgcctacctataaacccgtgaacccgtgtctgaaaaaaccgtgcaaatataacggcgtttgtaaaccgcgtggtggcagctacaagtgcttctgcaaaggtggttattacggctataactgcaatgcaaagccgacctacccgtcaacctataaggccaagccgagttatccaccgacctataaggcgaagccgagctatccgtcgacctacaagtaactcgagaaa

SEQ ID NO: 40 - DNA, 299 bp, synthetic construct(FP121-3 gene (gene fragment after vector insertion))
  source 1..299: mol_type = other DNA
tatggctaagagcagctacccgccaacgtacaaagcgaaaccgagctatccgccgacgtacaaggccaagccgtcctacccgcctacctataaacccgtgaacccgtgtctgaaaaaaccgtgcaaatataacggcgtttgtaaaccgcgtggtggcagctacaagtgcttctgcaaaggtggttattacggctataactgcaatgcaaagccgacctacccgtcaacctataaggccaagccgagttatccaccgacctataaggcgaagccgagctatccgtcgacctacaagtaac

SEQ ID NO: 41 - DNA, 42 bp, synthetic construct(FP121-3 gene Forward primer)
  source 1..42: mol_type = other DNA
aaacatatggctaagagcagctacccgccaacgtacaaagcg

SEQ ID NO: 42 - DNA, 37 bp, synthetic construct(FP121-3 gene reverse primer)
  source 1..37: mol_type = other DNA
tttctcgagttacttgtaggtcgacggatagctcggc

SEQ ID NO: 43 - DNA, 842 bp, synthetic construct((FP121-9 gene) (gene fragment after synthesis))
  source 1..842: mol_type = other DNA
taatacgactcactataggggaattgtgagcggataacaattcccctctagaaataattttgtttaactttaagaaggagatatacatatggctaaaccaacatatccctcaacttacaaggcgaagccgtcctacccgcctacttacaaggctaagccgtcttacccgtccacctacaaagccaagccgacgtacccctcaacttacaaggcgaagccgtcctacccgcctacttacaaggctaagccgtcttacccgtccacctacaaagctaagagcagctacccgccaacgtacaaagcgaaaccgagctatccgccgacgtacaaggccaagccgtcctacccgcctacctataaacccgtgaacccgtgtctgaaaaaaccgtgcaaatataacggcgtttgtaaaccgcgtggtggcagctacaagtgcttctgcaaaggtggttattacggctataactgcaatgcaaagccgacctacccgtcaacctataaggccaagccgagttatccaccgacctataaggcgaagccgagctatccgtcgacctacaaggcgaaaagcagctacccaccgacctataaagcgaaaccgagctatccgccgacctataaggcaaaaccgtcttacccgccgacatacaaagcgaaaagcagctacccaccgacctataaagcgaaaccgagctatccgccgacctataaggcaaaaccgtcttacccgccgacgtacaagtaactcgagcaccaccaccaccaccactgagatccggctgctaacaaagcccgaaaggaagctgagttggctgctgccaccgctgagcaataactagcat

SEQ ID NO: 44 - DNA, 292 bp, synthetic construct(Gene fragment A)
  source 1..292: mol_type = other DNA
gccaagccgacgtacccctcaacttacaaggcgaagccgtcctacccgcctacttacaaggctaagccgtcttacccgtccacctacaaagctaagagcagctacccgccaacgtacaaagcgaaaccgagctatccgccgacgtacaaggccaagccgtcctacccgcctacctataaacccgtgaacccgtgtctgaaaaaaccgtgcaaatataacggcgtttgtaaaccgcgtggtggcagctacaagtgcttctgcaaaggtggttattacggctataactgcaatg

SEQ ID NO: 45 - DNA, 292 bp, synthetic construct(Gene fragment B)
  source 1..292: mol_type = other DNA
cccgtgaacccgtgtctgaaaaaaccgtgcaaatataacggcgtttgtaaaccgcgtggtggcagctacaagtgcttctgcaaaggtggttattacggctataactgcaatgcaaagccgacctacccgtcaacctataaggccaagccgagttatccaccgacctataaggcgaagccgagctatccgtcgacctacaaggcgaaaagcagctacccaccgacctataaagcgaaaccgagctatccgccgacctataaggcaaaaccgtcttacccgccgacatacaaag

SEQ ID NO: 46 - DNA, 217 bp, synthetic construct(Gene fragment C)
  source 1..217: mol_type = other DNA
taatacgactcactataggggaattgtgagcggataacaattcccctctagaaataattttgtttaactttaagaaggagatatacatatggctaaaccaacatatccctcaacttacaaggcgaagccgtcctacccgcctacttacaaggctaagccgtcttacccgtccacctacaaagccaagccgacgtacccctcaacttacaaggcgaag

SEQ ID NO: 47 - DNA, 220 bp, synthetic construct(Gene fragment D)
  source 1..220: mol_type = other DNA
gcaaaaccgtcttacccgccgacatacaaagcgaaaagcagctacccaccgacctataaagcgaaaccgagctatccgccgacctataaggcaaaaccgtcttacccgccgacgtacaagtaactcgagcaccaccaccaccaccactgagatccggctgctaacaaagcccgaaaggaagctgagttggctgctgccaccgctgagcaataactagcat

SEQ ID NO: 48 - DNA, 36 bp, synthetic construct(FP121-9-Fragment-A Forward Primer)
  source 1..36: mol_type = other DNA
gccaagccgacgtacccctcaacttacaaggcgaag

SEQ ID NO: 49 - DNA, 25 bp, synthetic construct(FP121-9-Fragment-A Reverse Primer)
  source 1..25: mol_type = other DNA
cattgcagttatagccgtaataacc

SEQ ID NO: 50 - DNA, 18 bp, synthetic construct(FP121-9-Fragment-B Forward Primer)
  source 1..18: mol_type = other DNA
cccgtgaacccgtgtctg

SEQ ID NO: 51 - DNA, 31 bp, synthetic construct(FP121-9-Fragment-B Reverse Primer)
  source 1..31: mol_type = other DNA
ctttgtatgtcggcgggtaagacggttttgc

SEQ ID NO: 52 - DNA, 58 bp, synthetic construct(FP121-9-Fragment-C Reverse primer)
  source 1..58: mol_type = other DNA
cttcgccttgtaagttgaggggtacgtcggcttggctttgtaggtggacgggtaagac

SEQ ID NO: 53 - DNA, 50 bp, synthetic construct(FP121-9-Fragment-D Forward primer)
  source 1..50: mol_type = other DNA
gcaaaaccgtcttacccgccgacatacaaagcgaaaagcagctacccacc

SEQ ID NO: 54 - DNA, 21 bp, synthetic construct(T7 terminator reverse primer)
  source 1..21: mol_type = other DNA
atgctagttattgctcagcgg

SEQ ID NO: 55 - DNA, 473 bp, synthetic construct(Gene fragment AC)
  source 1..473: mol_type = other DNA
taatacgactcactataggggaattgtgagcggataacaattcccctctagaaataattttgtttaactttaagaaggagatatacatatggctaaaccaacatatccctcaacttacaaggcgaagccgtcctacccgcctacttacaaggctaagccgtcttacccgtccacctacaaagccaagccgacgtacccctcaacttacaaggcgaagccgtcctacccgcctacttacaaggctaagccgtcttacccgtccacctacaaagctaagagcagctacccgccaacgtacaaagcgaaaccgagctatccgccgacgtacaaggccaagccgtcctacccgcctacctataaacccgtgaacccgtgtctgaaaaaaccgtgcaaatataacggcgtttgtaaaccgcgtggtggcagctacaagtgcttctgcaaaggtggttattacggctataactgcaatg

SEQ ID NO: 56 - DNA, 481 bp, synthetic construct(Gene fragment BD)
  source 1..481: mol_type = other DNA
cccgtgaacccgtgtctgaaaaaaccgtgcaaatataacggcgtttgtaaaccgcgtggtggcagctacaagtgcttctgcaaaggtggttattacggctataactgcaatgcaaagccgacctacccgtcaacctataaggccaagccgagttatccaccgacctataaggcgaagccgagctatccgtcgacctacaaggcgaaaagcagctacccaccgacctataaagcgaaaccgagctatccgccgacctataaggcaaaaccgtcttacccgccgacatacaaagcgaaaagcagctacccaccgacctataaagcgaaaccgagctatccgccgacctataaggcaaaaccgtcttacccgccgacgtacaagtaactcgagcaccaccaccaccaccactgagatccggctgctaacaaagcccgaaaggaagctgagttggctgctgccaccgctgagcaataactagcat

SEQ ID NO: 57 - DNA, 659 bp, synthetic construct((FP121-9 gene) (gene fragment after vector insertion))
  source 1..659: mol_type = other DNA
tatggctaaaccaacatatccctcaacttacaaggcgaagccgtcctacccgcctacttacaaggctaagccgtcttacccgtccacctacaaagccaagccgacgtacccctcaacttacaaggcgaagccgtcctacccgcctacttacaaggctaagccgtcttacccgtccacctacaaagctaagagcagctacccgccaacgtacaaagcgaaaccgagctatccgccgacgtacaaggccaagccgtcctacccgcctacctataaacccgtgaacccgtgtctgaaaaaaccgtgcaaatataacggcgtttgtaaaccgcgtggtggcagctacaagtgcttctgcaaaggtggttattacggctataactgcaatgcaaagccgacctacccgtcaacctataaggccaagccgagttatccaccgacctataaggcgaagccgagctatccgtcgacctacaaggcgaaaagcagctacccaccgacctataaagcgaaaccgagctatccgccgacctataaggcaaaaccgtcttacccgccgacatacaaagcgaaaagcagctacccaccgacctataaagcgaaaccgagctatccgccgacctataaggcaaaaccgtcttacccgccgacgtacaagtaac

SEQ ID NO: 58 - DNA, 394 bp, synthetic construct(FP120 gene (gene fragment after synthesis))
  source 1..394: mol_type = other DNA
taatacgactcactataggggaattgtgagcggataacaattcccctctagaaataattttgtttaactttaagaaggagatatacatatggctaaaccaacatacccctcaacttacaaggcgaagccgtcctacccgcctacttacaaggctaagccgtcttacccgtccacctacaaagctaagagcagctacccgccaacgtacaaagcgaaaccgagctatccgccgacgtacaaggccaagccgtcctacccgcctacctataaacccgtgaacccgtgtctgaaaaaaccgtgcaaatataacggcgtttgtaaaccgcgtggtggcagctacaagtgcttctgcaaaggtggttattacggctataactgcaattaactcgagaaa

SEQ ID NO: 59 - DNA, 36 bp, synthetic construct(FP120 gene Reverse primer)
  source 1..36: mol_type = other DNA
tttctcgagttaattgcagttatagccgtaataacc

SEQ ID NO: 60 - DNA, 299 bp, synthetic construct(FP120 gene (gene fragment after vector insertion))
  source 1..299: mol_type = other DNA
tatggctaaaccaacatacccctcaacttacaaggcgaagccgtcctacccgcctacttacaaggctaagccgtcttacccgtccacctacaaagctaagagcagctacccgccaacgtacaaagcgaaaccgagctatccgccgacgtacaaggccaagccgtcctacccgcctacctataaacccgtgaacccgtgtctgaaaaaaccgtgcaaatataacggcgtttgtaaaccgcgtggtggcagctacaagtgcttctgcaaaggtggttattacggctataactgcaattaac

SEQ ID NO: 61 - DNA, 400 bp, synthetic construct(FP021 gene (gene fragment after synthesis))
  source 1..400: mol_type = other DNA
aaacatatgcccgtgaacccgtgtctgaaaaaaccgtgcaaatataacggcgtttgtaaaccgcgtggtggcagctacaagtgcttctgcaaaggtggttattacggctataactgcaatgcaaagccgacctacccgtcaacctataaggccaagccgagttatccaccgacctataaggcgaagccgagctatccgtcgacctacaaggcgaaaagcagctacccaccgacctataaagcgaaaccgagctatccgccgacctataaggcaaaaccgtcttacccgccgacgtacaagtaactcgagcaccaccaccaccaccactgagatccggctgctaacaaagcccgaaaggaagctgagttggctgctgccaccgctgagcaataactagcat

SEQ ID NO: 62 - DNA, 27 bp, synthetic construct(FP021 gene Forward primer)
  source 1..27: mol_type = other DNA
aaacatatgcccgtgaacccgtgtctg

SEQ ID NO: 63 - DNA, 299 bp, synthetic construct(FP021 gene (gene fragment after vector insertion))
  source 1..299: mol_type = other DNA
tatgcccgtgaacccgtgtctgaaaaaaccgtgcaaatataacggcgtttgtaaaccgcgtggtggcagctacaagtgcttctgcaaaggtggttattacggctataactgcaatgcaaagccgacctacccgtcaacctataaggccaagccgagttatccaccgacctataaggcgaagccgagctatccgtcgacctacaaggcgaaaagcagctacccaccgacctataaagcgaaaccgagctatccgccgacctataaggcaaaaccgtcttacccgccgacgtacaagtaac

SEQ ID NO: 64 - protein, 165 aa, FP121-6 (prototype) Amino acid sequence
MAKPTYPSTYKAKPSYPPTYKAKPSYPSTYKAKSSYPPTYKAKPSYPPTYKAKPSYPPTYKPVNPCLKKPCKYNGVCKPRGGSYKCFCKGGYYGYNCNAKPTYPSTYKAKPSYPPTYKAKPSYPSTYKAKSSYPPTYKAKPSYPPTYKAKPSYPPTYLEHHHHHH

SEQ ID NO: 65 - protein, 158 aa, FP121-6 Amino Acid Sequence
MAKPTYPSTYKAKPSYPPTYKAKPSYPSTYKAKSSYPPTYKAKPSYPPTYKAKPSYPPTYKPVNPCLKKPCKYNGVCKPRGGSYKCFCKGGYYGYNCNAKPTYPSTYKAKPSYPPTYKAKPSYPSTYKAKSSYPPTYKAKPSYPPTYKAKPSYPPTYK

SEQ ID NO: 66 - protein, 157 aa, cbFP121-6 Amino acid sequence
MAKPTYPSTYKAKPSYPPTYKAKPSYPSTYKAKSSYPPTYKAKPSYPPTYKAKPSYPPTYKKVNVCKPTPCKNSGRCVNKGSSYNCICKGGYSGPTCAKPTYPSTYKAKPSYPPTYKAKPSYPSTYKAKSSYPPTYKAKPSYPPTYKAKPSYPPTYK

SEQ ID NO: 67 - protein, 174 aa, hEGF-FP1-6 Amino acid sequence
MAKPTYPSTYKAKPSYPPTYKAKPSYPSTYKAKSSYPPTYKAKPSYPPTYKAKPSYPPTYKNSDSECPLSHDGYCLHDGVCMYIEALDKYACNCVVGYIGERCQYRDLKWWELRAKPTYPSTYKAKPSYPPTYKAKPSYPSTYKAKSSYPPTYKAKPSYPPTYKAKPSYPPTYK

SEQ ID NO: 68 - protein, 58 aa, FP121-1 Amino acid sequence
MAKPSYPPTYKPVNPCLKKPCKYNGVCKPRGGSYKCFCKGGYYGYNCNAKPTYPSTYK

SEQ ID NO: 69 - protein, 98 aa, FP121-3 Amino acid sequence
MAKSSYPPTYKAKPSYPPTYKAKPSYPPTYKPVNPCLKKPCKYNGVCKPRGGSYKCFCKGGYYGYNCNAKPTYPSTYKAKPSYPPTYKAKPSYPSTYK

SEQ ID NO: 70 - protein, 218 aa, FP121-9 Amino acid sequence
MAKPTYPSTYKAKPSYPPTYKAKPSYPSTYKAKPTYPSTYKAKPSYPPTYKAKPSYPSTYKAKSSYPPTYKAKPSYPPTYKAKPSYPPTYKPVNPCLKKPCKYNGVCKPRGGSYKCFCKGGYYGYNCNAKPTYPSTYKAKPSYPPTYKAKPSYPSTYKAKSSYPPTYKAKPSYPPTYKAKPSYPPTYKAKSSYPPTYKAKPSYPPTYKAKPSYPPTYK

SEQ ID NO: 71 - protein, 98 aa, FP120 Amino acid sequence
MAKPTYPSTYKAKPSYPPTYKAKPSYPSTYKAKSSYPPTYKAKPSYPPTYKAKPSYPPTYKPVNPCLKKPCKYNGVCKPRGGSYKCFCKGGYYGYNCN

SEQ ID NO: 72 - protein, 98 aa, FP021 Amino acid sequence
MPVNPCLKKPCKYNGVCKPRGGSYKCFCKGGYYGYNCNAKPTYPSTYKAKPSYPPTYKAKPSYPSTYKAKSSYPPTYKAKPSYPPTYKAKPSYPPTYK

SEQ ID NO: 73 - protein, 205 aa, FP151 Amino acid sequence
MAKPTYPSTYKAKPSYPPTYKAKPSYPSTYKAKSSYPPTYKAKPSYPPTYKAKPSYPPTYKSSEEYKGGYYPGNTYHYHSGGSYHGSGYHGGYKGKYYGKAKKYYYKYKNSGKYKYLKKARKYHRKGYKKYYGGGSSAKPTYPSTYKAKPSYPPTYKAKPSYPSTYKAKSSYPPTYKAKPSYPPTYKAKPSYPPTYKLEHHHHHH

SEQ ID NO: 74 - DNA, 593 bp, synthetic construct(FP151 gene sequence (after vector insertion))
  source 1..593: mol_type = other DNA
tatggccaaacctacatacccgagcacctataaagcgaaacctagctaccctccgacgtacaaggcaaaaccaagttacccgagcacctataaagctaagtcttcatacccgccaacatataaggccaaaccgagctatccacctacctataaagcgaagccctcctatccaccaacttataaatcgtcggaagagtataaaggcggttactatccgggaaatacctaccattatcattccggcggttcttatcacggatctggttaccatggtggctataaagggaagtactatggcaaggcaaagaaatattattataagtacaagaacagcgggaaatataagtatctgaagaaagcccgcaaatatcaccgtaaaggttacaagaagtattatggcggcggtagttctgcgaaaccgacatatccgtcaacttataaagcaaaaccgagttacccgcccacctataaagccaaaccctcgtatccgtcaacgtataaagcaaagtctagctacccgcctacgtataaggcgaagccctcgtatccaccgacgtacaaagccaaaccgagttacccaccgacctacaaac

SEQ ID NO: 75 - protein, 241 aa, hNGF-FP1-6 Amino acid sequence
MAKPTYPSTYKAKPSYPPTYKAKPSYPSTYKAKSSYPPTYKAKPSYPPTYKAKPSYPPTYKSSSHPIFHRGEFSVCDSVSVWVGDKTTATDIKGKEVMVLGEVNINNSVFKQYFFETKCRDPNPVDSGCRGIDSKHWNSYCTTTHTFVKALTMDGKQAAWRFIRIDTACVCVLSRKAVRRAAKPTYPSTYKAKPSYPPTYKAKPSYPSTYKAKSSYPPTYKAKPSYPPTYKAKPSYPPTYK

SEQ ID NO: 76 - DNA, 732 bp, hNGF-FP1-6 gene
  source 1..732: mol_type = other DNA
catatggctaaaccaacatatccctcaacttacaaggcgaaaccgtcgtacccgccgacgtacaaagctaagccgtcctatccgtctacctataaagcgaaaagctcttacccgccgacgtacaaggccaagccgtcctatccaccgacctacaaggcgaagccctcctatccgccgacgtacaagagcagcagccacccgattttccaccgtggtgaattcagcgtgtgcgatagtgtgagcgtgtgggttggcgataaaaccactgcgaccgatatcaaaggcaaagaggtgatggtgttgggcgaagtgaacatcaataactccgtctttaaacaatattttttcgaaaccaaatgtcgcgacccgaacccggtagacagcggttgtcgtggtattgactcgaaacattggaacagctattgtaccaccacgcacacctttgtgaaagcgttgaccatggatggtaaacaggcagcgtggcgtttcatccgcatcgacaccgcctgcgtttgcgtgctgagtcgcaaggcggttcgtcgcgcaaagccgacctacccgtcaacctataaggcgaagccgagctatccgccgacatacaaggctaagccgtcctatccgtctacctacaaggcgaaatccagctacccaccgacctacaaggcgaagccttcctacccgcctacttacaaggctaaaccatcatatccgccaacgtacaagtaactcgag

SEQ ID NO: 77 - protein, 275 aa, hbFGF-FP1-6 Amino acid sequence
MAKPTYPSTYKAKPSYPPTYKAKPSYPSTYKAKSSYPPTYKAKPSYPPTYKAKPSYPPTYKAAGSITTLPALPEDGGSGAFPPGHFKDPKRLYCKNGGFFLRIHPDGRVDGVREKSDPHIKLQLQAEERGVVSIKGVCANRYLAMKEDGRLLASKCVTDECFFFERLESNNYNTYRSRKYTSWYVALKRTGQYKLGSKTGPGQKAILFLPMSAKSAKPTYPSTYKAKPSYPPTYKAKPSYPSTYKAKSSYPPTYKAKPSYPPTYKAKPSYPPTYK

SEQ ID NO: 78 - DNA, 837 bp, hbFGF-FP1-6 gene
  source 1..837: mol_type = other DNA
catatggctaaaccaacttacccctcaacatataaggctaaaccgtcgtacccgccgacctacaaagcgaagccgtcatacccgtccacctataaagccaagagcagctacccgccgacttacaaggcgaaacctagctacccgccaacttacaaggcgaagccgtcctatccgccaacctacaaagcggcaggcagcatcaccaccctgccggcgctgccggaggacggcggctccggtgcgtttccgccgggtcatttcaaagacccgaaacgcctgtattgtaaaaacggtggttttttcctgaggattcacccggatggccgtgttgacggcgtgcgtgaaaaatccgatccgcacatcaaactccagctgcaagctgaggaacgtggtgtcgtgagcatcaagggtgtgtgcgcaaatcgttatctggcaatgaaagaagacggccgcttgctcgcgagcaagtgcgttaccgatgagtgctttttcttcgagcgcttggaaagcaataactataacacctatcgtagccgtaaatataccagctggtatgttgcattaaaacgcaccggccaatataagctgggttcgaaaaccggtccgggtcagaaagcgattctgtttttgccgatgagcgccaagagtgctaagccgacgtatccttctacgtacaaggcgaagcctagttacccaccgacctataaggccaagccgtcctacccgtctacgtacaaagcgaaaagctcttacccgccgacctacaaggctaagccgagctatccgccaacgtacaaggcgaagccgagctacccgccgacctataaataactcgag

SEQ ID NO: 79 - protein, 121 aa, hNGF Amino acid sequence
KSSSHPIFHRGEFSVCDSVSVWVGDKTTATDIKGKEVMVLGEVNINNSVFKQYFFETKCRDPNPVDSGCRGIDSKHWNSYCTTTHTFVKALTMDGKQAAWRFIRIDTACVCVLSRKAVRRA

SEQ ID NO: 80 - protein, 155 aa, hbFGF Amino acid sequence
KAAGSITTLPALPEDGGSGAFPPGHFKDPKRLYCKNGGFFLRIHPDGRVDGVREKSDPHIKLQLQAEERGVVSIKGVCANRYLAMKEDGRLLASKCVTDECFFFERLESNNYNTYRSRKYTSWYVALKRTGQYKLGSKTGPGQKAILFLPMSAKS